European Patent Application EP 4 403 576 A1, published July 24, 2024. Title: FcγRⅢa 선택적 결합력 향상 당화 Fc 변이체들. Applicant: 고려대학교 산학협력단. Application KR 10-2021-0124554, filed September 17, 2021. The sequence listing filed with the application follows.

SEQUENCE LISTING (65 sequences)

SEQ ID NO: 1 - protein, 113 aa, synthetic construct
PCPAPELLGGPSVFLLPPKIKDTLMISRTPEVTCVVVDVSHEDPEVKFNWYVDGVEVHNAKTKPPEEQYNSTLRVVSILTVLHQDWLNGKEYKCKVSNKALPLPEEKTISKAK

SEQ ID NO: 2 - protein, 113 aa, synthetic construct
PCPAPELLGGPDVFLFPPKIKDTLMISRTPEVTCVVVDVSHEDPEVKFNWYVDGVEVHNAKTKPREEQYNSTLRVVSILTVLHQDWLNGKEYKCKVSNKALPLPEEKTISKQK

SEQ ID NO: 3 - protein, 113 aa, synthetic construct
PCPAPELLGGPDVFLFPPKPKDTLMISRTPEVTCVVVDVSHEDPEVKFNWYVDGVEVHNAKTKPPEEQYNSTLRVVSVLTVLHQDWLNGKEYKCKVSNKALPLPIEKTISKQK

SEQ ID NO: 4 - protein, 113 aa, synthetic construct
PCPAPELLGGPSVFLLPPKIKDTLMISRTPEVTCVVVDVSHEDPEVKFNWYVDGVEVHNAKTKPPEEQYNSTLRVVSVLTVLHQDWLNGKEYKCKVSNKALPLPEEKTISKAK

SEQ ID NO: 5 - protein, 113 aa, synthetic construct
PCPAPELLGGPSVFLLPPKIKDTLMISRTPEVTCVVVDVSHEDPEVKFNWYVDGVEVHNAKTKPPEEQYNSTYRVVSVLTVLHQDWLNGKEYKCKVSNKALPLPEEKTISKQK

SEQ ID NO: 6 - protein, 113 aa, synthetic construct
PCPAPELLGGPSVFLLPPKIKDTLMISRTPEVTCVVVDVSHEDPEVKFNWYVDGVEVHNAKTKPPEEQYNSTLRVVSILTVLHQDWLNGKEYKCKVSNKALPLPEEKTISKQK

SEQ ID NO: 7 - protein, 113 aa, synthetic construct
PCPAPELLGGPSVFLLPPKIKDTLMISRTPEVTCVVVDVSHEDPEVKFNWYVDGVEVHNAKTKPPEEQYNSTLRVISILTVLHQDWLNGKEYKCKVSNKALPLPEEKTISKQK

SEQ ID NO: 8 - protein, 113 aa, synthetic construct
PCPAPELLGGPSVFLFPPKPKDTLMISRTPEVTCVVVDVSHEDPEVKFNWYVDGVEVHNAKTKPPEEQYNSTLRVVSILTVLHQDWLNGKEYKCKVSNKALPLPEEKTISKQK

SEQ ID NO: 9 - protein, 113 aa, synthetic construct
PCPAPELLGGPSVFLLPPKIKDTLVISRTPEVTCVVVDVSHEDPEVKFNWYVDGVEVHNAKTKPPEEQYNSTLRVVSILTVLHQDWLNGKEYKCKVSNKALPLPEEKTISKQK

SEQ ID NO: 10 - protein, 113 aa, synthetic construct
PCPAPELLGGPDVFLLPPKPKDTLMISRTPEVTCVVVDVSHEDPEVKFNWYVDGVEVHNAKTKPPEEQYNSTLRVVSILTVLHQDWLNGKEYKCKVSNKALPLPEEKTISKAK

SEQ ID NO: 11 - protein, 113 aa, synthetic construct
PCPAPELLGGPDVFLFPPKIKDTLMISRTPEVTCVVVDVSHEDPEVKFNWYVDGVEVHNAKTKPREEQYNSTYRVVSVLTVLHQDWLNGKEYKCKVSNKALPLPEEKTISKQK

SEQ ID NO: 12 - protein, 113 aa, synthetic construct
PCPAPELLGGPSVFLLPPKIKDTLMISRTPEVTCVVVDVSHEDPEVKFNWYVDGVEVHNAKTKPPEEQYNSTLRVVSILTVLHQDWLNGKEYKCKVSNKALPAPIEKTISKQK

SEQ ID NO: 13 - protein, 113 aa, synthetic construct
PCPAPELLGGPDVFLLPPKIKDTLMISRTPEVTCVVVDVSHEDPEVKFNWYVDGVEVHNAKTKPPEEQYNSTLRVVSILTVLHQDWLNGKEYKCKVSNKALPLPEEKTISKQK

SEQ ID NO: 14 - protein, 107 aa, synthetic construct
GQPREPQVYTLPPSRDELTKDQVSLTCLVKGFYPSDIAVEWESNGQQENNYKTTPPVLDSDGSFFLYSKLTVDKSRWQQGNVFSCSVMHEALHNHYTQKSLSLSPGK

SEQ ID NO: 15 - protein, 107 aa, synthetic construct
GQPREPQVYTLPPSRDELTKNQVSLTCLVKGFYPSDIAVEWESNGQQENNYKTTPPVLDSDGSFLLYSKLTVDKSRWQQGNVFSCSVMHEALHNHYTQKSLSLSPGK

SEQ ID NO: 16 - protein, 107 aa, synthetic construct
GQPREPQVYTLPPSRDELTKNQVSLTCLVKGFYPSDIAVEWESNGQPENNYKTTPLVLDSDGSFFLYSKLTVDKSRWQQGNVFSCSVMHEALHNHYTQKSLSLSPGK

SEQ ID NO: 17 - protein, 107 aa, synthetic construct
GQPREPQVYTLPPSRDELTKNQVSLTCLVKGFYPSDIAVEWESNGQPENNYKTTPLVLDSDGSFFLYSKLTVDKGRWQQGNVFSCSVMHEALHNHYTQKSLSLSPGK

SEQ ID NO: 18 - protein, 107 aa, synthetic construct
GQPREPQVYTLPPSRDELTKNQVSLTCLVKGFYPSDIAVEWESNGQQENNYKTTPPVLDSDGSFFLYSKLTVDKSRWQQGNVFSCSVMHEALHNHYTQKSLSLSPGK

SEQ ID NO: 19 - protein, 107 aa, synthetic construct
GQPREPQVYTLPPSRGELTKNQVSLTCLVKGFYPSDIAVEWESNGQQENNYKTTPPVLDSDGSFFLYSKLTVDKSRWQQGNVFSCSVMHEALHNHYTQKSLSLSPGK

SEQ ID NO: 20 - protein, 107 aa, synthetic construct
GQPREPQVYTLPPSRDELTKNQVSLTCLVKGFYPSDIAVEWESNGQPENNYKTTPPVLDSDGSFFLYSKLTVDKSRWQQGNVFSCSVMHEALHNHYTQKSLSLSPGK

SEQ ID NO: 21 - protein, 227 aa, synthetic construct
DKTHTCPPCPAPELLGGPSVFLFPPKPKDTLMISRTPEVTCVVVDVSHEDPEVKFNWYVDGVEVHNAKTKPREEQYNSTYRVVSVLTVLHQDWLNGKEYKCKVSNKALPAPIEKTISKAKGQPREPQVYTLPPSRDELTKNQVSLTCLVKGFYPSDIAVEWESNGQPENNYKTTPPVLDSDGSFFLYSKLTVDKSRWQQGNVFSCSVMHEALHNHYTQKSLSLSPGK

SEQ ID NO: 22 - protein, 227 aa, synthetic construct
DNTHTCPPCPAPELLGGPSVFLLPPKIKDTLMISRTPEVTCVVVDVSHEDPEVKFNWYVDGVEVHNAKTKPPEEQYNSTLRVVSILTVLHQDWLNGKEYKCKVSNKALPLPEEKTISKAKGQPREPQVYTLPPSRDELTKNQVSLTCLVKGFYPSDIAVEWESNGQPENNYKTTPPVLDSDGSFFLYSKLTVDKSRWQQGNVFSCSVMHEALHNHYTQKSLSLSPGK

SEQ ID NO: 23 - protein, 227 aa, synthetic construct
DKTHTCPPCPAPELLGGPDVFLFPPKIKDTLMISRTPEVTCVVVDVSHEDPEVKFNWYVDGVEVHNAKTKPREEQYNSTLRVVSILTVLHQDWLNGKEYKCKVSNKALPLPEEKTISKQKGQPREPQVYTLPPSRDELTKDQVSLTCLVKGFYPSDIAVEWESNGQQENNYKTTPPVLDSDGSFFLYSKLTVDKSRWQQGNVFSCSVMHEALHNHYTQKSLSLSPGK

SEQ ID NO: 24 - protein, 227 aa, synthetic construct
DKTHTCPPCPAPELLGGPDVFLFPPKPKDTLMISRTPEVTCVVVDVSHEDPEVKFNWYVDGVEVHNAKTKPPEEQYNSTLRVVSVLTVLHQDWLNGKEYKCKVSNKALPLPIEKTISKQKGQPREPQVYTLPPSRDELTKNQVSLTCLVKGFYPSDIAVEWESNGQQENNYKTTPPVLDSDGSFLLYSKLTVDKSRWQQGNVFSCSVMHEALHNHYTQKSLSLSPGK

SEQ ID NO: 25 - protein, 227 aa, synthetic construct
DKTHTCPPCPAPELLGGPSVFLLPPKIKDTLMISRTPEVTCVVVDVSHEDPEVKFNWYVDGVEVHNAKTKPPEEQYNSTLRVVSVLTVLHQDWLNGKEYKCKVSNKALPLPEEKTISKAKGQPREPQVYTLPPSRDELTKNQVSLTCLVKGFYPSDIAVEWESNGQPENNYKTTPLVLDSDGSFFLYSKLTVDKSRWQQGNVFSCSVMHEALHNHYTQKSLSLSPGK

SEQ ID NO: 26 - protein, 227 aa, synthetic construct
DKTHTCPPCPAPELLGGPSVFLLPPKIKDTLMISRTPEVTCVVVDVSHEDPEVKFNWYVDGVEVHNAKTKPPEEQYNSTYRVVSVLTVLHQDWLNGKEYKCKVSNKALPLPEEKTISKQKGQPREPQVYTLPPSRDELTKNQVSLTCLVKGFYPSDIAVEWESNGQPENNYKTTPLVLDSDGSFFLYSKLTVDKGRWQQGNVFSCSVMHEALHNHYTQKSLSLSPGK

SEQ ID NO: 27 - protein, 227 aa, synthetic construct
DKTHTCPPCPAPELLGGPSVFLLPPKIKDTLMISRTPEVTCVVVDVSHEDPEVKFNWYVDGVEVHNAKTKPPEEQYNSTLRVVSILTVLHQDWLNGKEYKCKVSNKALPLPEEKTISKQKGQPREPQVYTLPPSRDELTKNQVSLTCLVKGFYPSDIAVEWESNGQQENNYKTTPPVLDSDGSFFLYSKLTVDKSRWQQGNVFSCSVMHEALHNHYTQKSLSLSPGK

SEQ ID NO: 28 - protein, 227 aa, synthetic construct
DKTRTCPPCPAPELLGGPSVFLLPPKIKDTLMISRTPEVTCVVVDVSHEDPEVKFNWYVDGVEVHNAKTKPPEEQYNSTLRVISILTVLHQDWLNGKEYKCKVSNKALPLPEEKTISKQKGQPREPQVYTLPPSRDELTKNQVSLTCLVKGFYPSDIAVEWESNGQQENNYKTTPPVLDSDGSFFLYSKLTVDKSRWQQGNVFSCSVMHEALHNHYTQKSLSLSPGK

SEQ ID NO: 29 - protein, 227 aa, synthetic construct
DKTHTCPPCPAPELLGGPSVFLFPPKPKDTLMISRTPEVTCVVVDVSHEDPEVKFNWYVDGVEVHNAKTKPPEEQYNSTLRVVSILTVLHQDWLNGKEYKCKVSNKALPLPEEKTISKQKGQPREPQVYTLPPSRDELTKNQVSLTCLVKGFYPSDIAVEWESNGQQENNYKTTPPVLDSDGSFFLYSKLTVDKSRWQQGNVFSCSVMHEALHNHYTQKSLSLSPGK

SEQ ID NO: 30 - protein, 227 aa, synthetic construct
DKTHTCPPCPAPELLGGPSVFLLPPKIKDTLVISRTPEVTCVVVDVSHEDPEVKFNWYVDGVEVHNAKTKPPEEQYNSTLRVVSILTVLHQDWLNGKEYKCKVSNKALPLPEEKTISKQKGQPREPQVYTLPPSRGELTKNQVSLTCLVKGFYPSDIAVEWESNGQQENNYKTTPPVLDSDGSFFLYSKLTVDKSRWQQGNVFSCSVMHEALHNHYTQKSLSLSPGK

SEQ ID NO: 31 - protein, 227 aa, synthetic construct
DKTHTCPPCPAPELLGGPSVFLLPPKIKDTLMISRTPEVTCVVVDVSHEDPEVKFNWYVDGVEVHNAKTKPPEEQYNSTLRVVSILTVLHQDWLNGKEYKCKVSNKALPLPEEKTISKQKGQPREPQVYTLPPSRGELTKNQVSLTCLVKGFYPSDIAVEWESNGQQENNYKTTPPVLDSDGSFFLYSKLTVDKSRWQQGNVFSCSVMHEALHNHYTQKSLSLSPGK

SEQ ID NO: 32 - protein, 227 aa, synthetic construct
DKTHTCPPCPAPELLGGPDVFLLPPKPKDTLMISRTPEVTCVVVDVSHEDPEVKFNWYVDGVEVHNAKTKPPEEQYNSTLRVVSILTVLHQDWLNGKEYKCKVSNKALPLPEEKTISKAKGQPREPQVYTLPPSRDELTKNQVSLTCLVKGFYPSDIAVEWESNGQPENNYKTTPLVLDSDGSFFLYSKLTVDKSRWQQGNVFSCSVMHEALHNHYTQKSLSLSPGK

SEQ ID NO: 33 - protein, 227 aa, synthetic construct
DKTHTCPPCPAPELLGGPDVFLFPPKIKDTLMISRTPEVTCVVVDVSHEDPEVKFNWYVDGVEVHNAKTKPREEQYNSTYRVVSVLTVLHQDWLNGKEYKCKVSNKALPLPEEKTISKQKGQPREPQVYTLPPSRDELTKNQVSLTCLVKGFYPSDIAVEWESNGQPENNYKTTPPVLDSDGSFFLYSKLTVDKSRWQQGNVFSCSVMHEALHNHYTQKSLSLSPGK

SEQ ID NO: 34 - protein, 227 aa, synthetic construct
DKTHTCPPCPAPELLGGPSVFLLPPKIKDTLMISRTPEVTCVVVDVSHEDPEVKFNWYVDGVEVHNAKTKPPEEQYNSTLRVVSILTVLHQDWLNGKEYKCKVSNKALPAPIEKTISKQKGQPREPQVYTLPPSRDELTKNQVSLTCLVKGFYPSDIAVEWESNGQPENNYKTTPLVLDSDGSFFLYSKLTVDKSRWQQGNVFSCSVMHEALHNHYTQKSLSLSPGK

SEQ ID NO: 35 - protein, 227 aa, synthetic construct
DKTHTCPPCPAPELLGGPDVFLLPPKIKDTLMISRTPEVTCVVVDVSHEDPEVKFNWYVDGVEVHNAKTKPPEEQYNSTLRVVSILTVLHQDWLNGKEYKCKVSNKALPLPEEKTISKQKGQPREPQVYTLPPSRDELTKNQVSLTCLVKGFYPSDIAVEWESNGQPENNYKTTPLVLDSDGSFFLYSKLTVDKSRWQQGNVFSCSVMHEALHNHYTQKSLSLSPGK

SEQ ID NO: 36 - DNA, 681 bp, synthetic construct
  source 1..681: mol_type = other DNA
gacaaaactcacacatgcccaccgtgcccagcacctgaactcctggggggaccgtcagtcttcctcttccccccaaaacccaaggacaccctcatgatctcccggacccctgaggtcacatgcgtggtggtggacgtgagccacgaagaccctgaggtcaagttcaactggtacgtggacggcgtggaggtgcataatgccaagacaaagccgcgggaggagcagtacaacagcacgtaccgtgtggtcagcgtcctcaccgtcctgcaccaggactggctgaatggcaaggagtacaagtgcaaggtctccaacaaagccctcccagcccccatcgagaaaaccatctccaaagccaaagggcagccccgagaaccacaggtgtacaccctgcccccatcccgggatgagctgaccaagaaccaggtcagcctgacctgcctggtcaaaggcttctatcccagcgacatcgccgtggagtgggagagcaatgggcagccggagaacaactacaagaccacacctcccgtgctggactccgacggctccttcttcctctacagcaagctcaccgtggacaagagcaggtggcagcaggggaacgtcttctcatgctccgtgatgcatgaggctctgcacaaccactacacgcagaagagcctctccctgtccccgggtaaa

SEQ ID NO: 37 - DNA, 681 bp, synthetic construct
  source 1..681: mol_type = other DNA
gacaatactcacacatgcccaccgtgcccagcacctgaactcctggggggaccgtcagtcttcctcctccccccaaaaatcaaggacaccctcatgatctcccggacccctgaggtcacatgcgtggtggtggacgtgagccacgaagaccctgaggtcaagttcaactggtacgtggacggcgtggaggtgcataatgccaagacaaagccgcccgaggagcagtacaacagcacgctgcgtgtggtcagcattctcaccgtcctgcaccaggactggctgaatggcaaggagtacaagtgcaaggtctccaacaaagccctcccactgcccgaggagaaaaccatctccaaagccaaagggcagccccgagaaccacaggtgtacaccctgcccccatcccgggatgagctgaccaagaaccaggtcagcctgacctgcctggtcaaaggcttctatcccagcgacatcgccgtggagtgggagagcaatgggcagccggagaacaactacaagaccacgcctcccgtgctggactccgacggctccttcttcctctacagcaagctcaccgtggacaagagcaggtggcagcaggggaacgtcttctcatgctccgtgatgcatgaggctctgcacaaccactacacgcagaagagcctctccctgtccccgggtaaa

SEQ ID NO: 38 - DNA, 681 bp, synthetic construct
  source 1..681: mol_type = other DNA
gacaaaactcacacatgcccaccgtgcccagcacctgaactcctggggggaccggacgtcttcctcttccccccaaaaatcaaggacaccctcatgatctcccggacccctgaggtcacatgcgtggtggtggacgtgagccacgaagaccctgaggtcaagttcaactggtacgtggacggcgtggaggtgcataatgccaagacaaagccgcgtgaggagcagtacaacagcacgctgcgtgtggtcagcattctcaccgtcctgcaccaggactggctgaatggcaaggagtacaagtgcaaggtctccaacaaagccctcccactgcccgaggagaaaaccatctccaaacagaaagggcagccccgagaaccacaggtgtacaccctgcccccatcccgggatgagctgaccaaggaccaggtcagcctgacctgcctggtcaaaggcttctatcccagcgacatcgccgtggagtgggagagcaatgggcagcaggagaacaactacaagaccacgcctcccgtgctggactccgacggctccttcttcctctacagcaagctcaccgtggacaagagcaggtggcagcaggggaacgtcttctcatgctccgtgatgcatgaggctctgcacaaccactacacgcagaagagcctctccctgtccccgggtaaa

SEQ ID NO: 39 - DNA, 681 bp, synthetic construct
  source 1..681: mol_type = other DNA
gacaaaactcacacatgcccaccgtgcccagcacctgaactcctggggggaccggacgtcttcctcttccccccaaaacccaaggacaccctcatgatctcccggacccctgaggtcacatgcgtggtggtggacgtgagccacgaagaccctgaggtcaagttcaactggtacgtggacggcgtggaggtgcataatgccaagacaaagccgcccgaggagcagtacaacagcacgctgcgtgtggtcagcgtcctcaccgtcctgcaccaggactggctgaatggcaaggagtacaagtgcaaggtctccaacaaagccctcccactgcccatcgagaaaaccatctccaaacagaaagggcagccccgagaaccacaggtgtacaccctgcccccatcccgggatgagctgaccaagaaccaggtcagcctgacctgcctggtcaaaggcttctatcccagcgacatcgccgtggagtgggagagcaatgggcagcaggagaacaactacaagaccacgcctcccgtgctggactccgacggctccttcctcctctacagcaagctcaccgtggacaagagcaggtggcagcaggggaacgtcttctcatgctccgtgatgcatgaggctctgcacaaccactacacgcagaagagcctctccctgtccccgggtaaa

SEQ ID NO: 40 - DNA, 681 bp, synthetic construct
  source 1..681: mol_type = other DNA
gacaaaactcacacatgcccaccgtgcccagcacctgaactcctggggggaccgtcagtcttcctccttcccccaaaaatcaaggacaccctcatgatctcccggacccctgaggtcacatgcgtggtggtggacgtgagccacgaagaccctgaggtcaagttcaactggtacgtggacggcgtggaggtgcataatgccaagacaaagccgcctgaggagcagtacaacagcacgctgcgtgtggtcagcgttctcaccgtcctgcaccaggactggctgaatggcaaggagtacaagtgcaaggtctccaacaaagccctcccactgcccgaggagaaaaccatctccaaagccaaagggcagccccgagaaccacaggtgtacaccctgcccccatcccgggatgagctgaccaagaaccaggtcagcctgacctgcctggtcaaaggcttctatcccagcgacatcgccgtggagtgggagagcaatgggcagccggagaacaactacaagaccacgcctctggtgctggactccgacggctccttcttcctctacagcaagctcaccgtggacaagagcaggtggcagcaggggaacgtcttctcatgctccgtgatgcatgaggctctgcacaaccactacacgcagaagagcctctccctgtccccgggtaaa

SEQ ID NO: 41 - DNA, 681 bp, synthetic construct
  source 1..681: mol_type = other DNA
gacaaaactcacacatgcccaccgtgcccagcacctgaactcctggggggaccgtcagtcttcctccttcccccaaaaatcaaggacaccctcatgatctcccggacccctgaggtcacatgcgtggtggtggacgtgagccacgaagaccctgaggtcaagttcaactggtacgtggacggcgtggaggtgcataatgccaagacaaagccgcctgaggagcagtacaacagcacgtaccgtgtggtcagcgttctcaccgtcctgcaccaggactggctgaatggcaaggagtacaagtgcaaggtctccaacaaagccctcccactgcccgaggagaaaaccatctccaaacagaaagggcagccccgagaaccacaggtgtacaccctgcccccatcccgggatgagctgaccaagaaccaggtcagcctgacctgcctggtcaaaggcttctatcccagcgacatcgccgtggagtgggagagcaatgggcagccggagaacaactacaagaccacgcctctggtgctggactccgacggctctttcttcctctacagcaagctcaccgtggacaagggcaggtggcagcaggggaacgtcttctcatgctccgtgatgcatgaggctctgcacaaccactacacgcagaagagcctctccctgtccccgggtaaa

SEQ ID NO: 42 - DNA, 681 bp, synthetic construct
  source 1..681: mol_type = other DNA
gacaaaactcacacatgcccaccgtgcccagcacctgaactcctggggggaccgtcagtcttcctcctccccccaaaaatcaaggacaccctcatgatctcccggacccctgaggtcacatgcgtggtggtggacgtgagccacgaagaccctgaggtcaagttcaactggtacgtggacggcgtggaggtgcataatgccaagacaaagccgcctgaggagcagtacaacagcacgctgcgtgtggtcagcattctcaccgtcctgcaccaggactggctgaatggcaaggagtacaagtgcaaggtctccaacaaagccctcccactgcccgaggagaaaaccatctccaaacagaaagggcagccccgagaaccacaggtgtacaccctgcccccatcccgggatgagctgaccaagaaccaggtcagcctgacctgcctggtcaaaggcttctatcccagcgacatcgccgtggagtgggagagcaatgggcagcaggagaacaactacaagaccacgcctcccgtgctggactccgacggctccttcttcctctacagcaagctcaccgtggacaagagcaggtggcagcaggggaacgtcttctcatgctccgtgatgcatgaggctctgcacaaccactacacgcagaagagcctctccctgtccccgggtaaa

SEQ ID NO: 43 - DNA, 681 bp, synthetic construct
  source 1..681: mol_type = other DNA
gacaaaactcgcacatgcccaccgtgcccagcacctgaactcctggggggaccgtcagtcttcctcctccccccaaaaatcaaggacaccctcatgatctcccggacccctgaggtcacatgcgtggtggtggacgtgagccacgaagaccctgaggtcaagttcaactggtacgtggacggcgtggaggtgcataatgccaagacaaagccgcctgaggagcagtacaacagcacgctgcgtgtgatcagcattctcaccgtcctgcaccaggactggctgaatggcaaggagtacaagtgcaaggtctccaacaaagccctcccactgcccgaggagaaaaccatctccaaacagaaagggcagccccgagaaccacaggtgtacaccctgcccccatcccgggatgagctgaccaagaaccaggtcagcctgacctgcctggtcaaaggcttctatcccagcgacatcgccgtggagtgggagagcaatgggcagcaggagaacaactacaagaccacgcctcccgtgctggactccgacggctccttcttcctctacagcaagctcaccgtggacaagagcaggtggcagcaggggaacgtcttctcatgctccgtgatgcatgaggctctgcacaaccactacacgcagaagagcctctccctgtccccgggtaaa

SEQ ID NO: 44 - DNA, 681 bp, synthetic construct
  source 1..681: mol_type = other DNA
gacaaaactcacacatgcccaccgtgcccagcacctgaactcctggggggaccgtcagtcttcctcttccccccaaaacccaaggacaccctcatgatctcccggacccctgaggtcacatgcgtggtggtggacgtgagccacgaagaccctgaggtcaagttcaactggtacgtggacggcgtggaggtgcataatgccaagacaaagccgcctgaggagcagtacaacagcacgctgcgtgtggtcagcattctcaccgtcctgcaccaggactggctgaatggcaaggagtacaagtgcaaggtctccaacaaagccctcccactgcccgaggagaaaaccatctccaaacagaaagggcagccccgagaaccacaggtgtacaccctgcccccatcccgggatgagctgaccaagaaccaggtcagcctgacctgcctggtcaaaggcttctatcccagcgacatcgccgtggagtgggagagcaatgggcagcaggagaacaactacaaaaccacgcctcccgtgctggactccgacggctccttcttcctctacagcaagctcaccgtggacaagagcaggtggcagcaggggaacgtcttctcatgctccgtgatgcatgaggctctgcacaaccactacacgcagaagagcctctccctgtccccgggtaaa

SEQ ID NO: 45 - DNA, 681 bp, synthetic construct
  source 1..681: mol_type = other DNA
gacaaaactcacacatgcccaccgtgcccagcacctgaactcctggggggaccgtcagtcttcctcctccccccaaaaatcaaggacaccctcgtgatctcccggacccctgaggtcacatgcgtggtggtggacgtgagccacgaagaccctgaggtcaagttcaactggtacgtggacggcgtggaggtgcataatgccaagacaaagccgcctgaggagcagtacaacagcacgctgcgcgtggtcagcattctcaccgtcctgcaccaggactggctgaatggcaaggagtacaagtgcaaggtctccaacaaagccctcccactgcccgaggagaaaaccatctccaaacagaaagggcagccccgagaaccacaggtgtacaccctgcccccatcccggggtgagctgaccaagaaccaggtcagcctgacctgcctggtcaaaggcttctatcccagcgacatcgccgtggagtgggagagcaatgggcagcaggagaacaactacaagaccacgcctcccgtgctggactccgacggctccttcttcctctacagcaagctcaccgtggacaagagcaggtggcagcaggggaacgtcttctcatgctccgtgatgcatgaggctctgcacaaccactacacgcagaagagcctctccctgtccccgggtaaa

SEQ ID NO: 46 - DNA, 681 bp, synthetic construct
  source 1..681: mol_type = other DNA
gacaaaactcacacatgcccaccgtgcccagcacctgaactcctggggggaccgtcagtcttcctcctccccccaaaaatcaaggacaccctcatgatctcccggacccctgaggtcacatgcgtggtggtggacgtgagccacgaagaccctgaggtcaagttcaactggtacgtggacggcgtggaggtgcataatgccaagacaaagccgcctgaggagcagtacaacagcacgctgcgtgtggtcagcattctcaccgtcctgcaccaggactggctgaatggcaaggagtacaagtgcaaggtctccaacaaagccctcccactgcccgaggagaaaaccatctccaaacagaaagggcagccccgagaaccacaggtgtacaccctgcccccatcccggggtgagctgaccaagaaccaggtcagcctgacctgcctggtcaaaggcttctatcccagcgacatcgccgtggagtgggagagcaatgggcagcaggagaacaactacaagaccacgcctcccgtgctggactccgacggctccttcttcctctacagcaagctcaccgtggacaagagcaggtggcagcaggggaacgtcttctcatgctccgtgatgcatgaggctctgcacaaccactacacgcagaagagcctctccctgtccccgggtaaa

SEQ ID NO: 47 - DNA, 681 bp, synthetic construct
  source 1..681: mol_type = other DNA
gacaaaactcacacatgcccaccgtgcccagcacctgaactcctggggggaccggacgtcttcctcctgcccccaaaacccaaggacaccctcatgatctcccggacccctgaggtcacatgcgtggtggtggacgtgagccacgaagaccctgaggtcaagttcaactggtacgtggacggcgtggaggtgcataatgccaagacaaagccgcccgaggagcagtacaacagcacgctgcgtgtggtcagcatcctcaccgtcctgcaccaggactggctgaatggcaaggagtacaagtgcaaggtctccaacaaagccctcccactgcccgaggagaaaaccatctccaaagccaaagggcagccccgagaaccacaggtgtacaccctgcccccatcccgggacgagctgaccaagaaccaggtcagcctgacctgcctggtcaaaggcttctatcccagcgacatcgccgtggagtgggagagcaatgggcagccggagaacaactacaagaccacgcctctggtgctggactccgacggctccttcttcctctacagcaagctcaccgtggacaagagcaggtggcagcaggggaacgtcttctcatgctccgtgatgcatgaggctctgcacaaccactacacgcagaagagcctctccctgtctccgggtaaa

SEQ ID NO: 48 - DNA, 681 bp, synthetic construct
  source 1..681: mol_type = other DNA
gacaaaactcacacatgcccaccgtgcccagcacctgaactcctggggggaccggacgtcttcctcttccccccaaaaatcaaggacaccctcatgatctcccggacccctgaggtcacatgcgtggtggtggacgtgagccacgaagaccctgaggtcaagttcaactggtacgtggacggcgtggaggtgcataatgccaagacaaagccgcgggaggagcagtacaacagcacgtaccgtgtggtcagcgtcctcaccgtcctgcaccaggactggctgaatggcaaggagtacaagtgcaaggtctccaacaaagccctcccactgcccgaggagaaaaccatctccaaacagaaagggcagccccgagaaccacaggtgtacaccctgcccccatcccgggacgagctgaccaagaaccaggtcagcctgacctgcctggtcaaaggcttctatcccagcgacatcgccgtggagtgggagagcaatgggcagccggagaacaactacaagaccacgcctcccgtgctggactccgacggctccttcttcctctacagcaagctcaccgtggacaagagcaggtggcagcaggggaacgtcttctcatgctccgtgatgcatgaggctctgcacaaccactacacgcagaagagcctctccctgtctccgggtaaa

SEQ ID NO: 49 - DNA, 681 bp, synthetic construct
  source 1..681: mol_type = other DNA
gacaaaactcacacatgcccaccgtgcccagcacctgaactcctggggggaccgtcagtcttcctcctgcccccaaaaatcaaggacaccctcatgatctcccggacccctgaggtcacatgcgtggtggtggacgtgagccacgaagaccctgaggtcaagttcaactggtacgtggacggcgtggaggtgcataatgccaagacaaagccgcccgaggagcagtacaacagcacgctgcgtgtggtcagcatcctcaccgtcctgcaccaggactggctgaatggcaaggagtacaagtgcaaggtctccaacaaagccctcccagcccccatcgagaaaaccatctccaaacagaaagggcagccccgagaaccacaggtgtacaccctgcccccatcccgggacgagctgaccaagaaccaggtcagcctgacctgcctggtcaaaggcttctatcccagcgacatcgccgtggagtgggagagcaatgggcagccggagaacaactacaagaccacgcctctggtgctggactccgacggctccttcttcctctacagcaagctcaccgtggacaagagcaggtggcagcaggggaacgtcttctcatgctccgtgatgcatgaggctctgcacaaccactacacgcagaagagcctctccctgtctccgggtaaa

SEQ ID NO: 50 - DNA, 681 bp, synthetic construct
  source 1..681: mol_type = other DNA
gacaaaactcacacatgcccaccgtgcccagcacctgaactcctggggggaccggacgtcttcctcctgcccccaaaaatcaaggacaccctcatgatctcccggacccctgaggtcacatgcgtggtggtggacgtgagccacgaagaccctgaggtcaagttcaactggtacgtggacggcgtggaggtgcataatgccaagacaaagccgcccgaggagcagtacaacagcacgctgcgtgtggtcagcatcctcaccgtcctgcaccaggactggctgaatggcaaggagtacaagtgcaaggtctccaacaaagccctcccactgcccgaggagaaaaccatctccaaacagaaagggcagccccgagaaccacaggtgtacaccctgcccccatcccgggacgagctgaccaagaaccaggtcagcctgacctgcctggtcaaaggcttctatcccagcgacatcgccgtggagtgggagagcaatgggcagccggagaacaactacaagaccacgcctctggtgctggactccgacggctccttcttcctctacagcaagctcaccgtggacaagagcaggtggcagcaggggaacgtcttctcatgctccgtgatgcatgaggctctgcacaaccactacacgcagaagagcctctccctgtctccgggtaaa

SEQ ID NO: 51 - protein, 214 aa, synthetic construct
DIQMTQSPSSLSASVGDRVTITCRASQDVNTAVAWYQQKPGKAPKLLIYSASFLYSGVPSRFSGSRSGTDFTLTISSLQPEDFATYYCQQHYTTPPTFGQGTKVEIKRTAAAPSVFIFPPSDEQLKSGTASVVCLLNNFYPREAKVQWKVDNALQSGNSQESVTEQDSKDSTYSLSSTLTLSKADYEKHKVYACEVTHQGLSSPVTKSFNRGEC

SEQ ID NO: 52 - protein, 451 aa, synthetic construct
EVQLVESGGGLVQPGGSLRLSCAASGFNIKDTYIHWVRQAPGKGLEWVARIYPTNGYTRYADSVKGRFTISADTSKNTAYLQMNSLRAEDTAVYYCSRWGGDGFYAMDYWGQGTLVTVSSASTKGPSVFPLAPSSKSTSGGTAALGCLVKDYFPEPVTVSWNSGALTSGVHTFPAVLQSSGLYSLSSVVTVPSSSLGTQTYICNVNHKPSNTKVDKKVEPPKSCDKTHTCPPCPAPELLGGPSVFLFPPKPKDTLMISRTPEVTCVVVDVSHEDPEVKFNWYVDGVEVHNAKTKPREEQYNSTYRVVSVLTVLHQDWLNGKEYKCKVSNKALPAPIEKTISKAKGQPREPQVYTLPPSRDELTKNQVSLTCLVKGFYPSDIAVEWESNGQPENNYKTTPPVLDSDGSFFLYSKLTVDKSRWQQGNVFSCSVMHEALHNHYTQKSLSLSPGK

SEQ ID NO: 53 - protein, 451 aa, synthetic construct
EVQLVESGGGLVQPGGSLRLSCAASGFNIKDTYIHWVRQAPGKGLEWVARIYPTNGYTRYADSVKGRFTISADTSKNTAYLQMNSLRAEDTAVYYCSRWGGDGFYAMDYWGQGTLVTVSSASTKGPSVFPLAPSSKSTSGGTAALGCLVKDYFPEPVTVSWNSGALTSGVHTFPAVLQSSGLYSLSSVVTVPSSSLGTQTYICNVNHKPSNTKVDKKVEPPKSCDKTHTCPPCPAPELLGGPSVFLLPPKIKDTLMISRTPEVTCVVVDVSHEDPEVKFNWYVDGVEVHNAKTKPPEEQYNSTLRVVSILTVLHQDWLNGKEYKCKVSNKALPLPEEKTISKQKGQPREPQVYTLPPSRDELTKNQVSLTCLVKGFYPSDIAVEWESNGQQENNYKTTPPVLDSDGSFFLYSKLTVDKSRWQQGNVFSCSVMHEALHNHYTQKSLSLSPGK

SEQ ID NO: 54 - protein, 451 aa, synthetic construct
EVQLVESGGGLVQPGGSLRLSCAASGFNIKDTYIHWVRQAPGKGLEWVARIYPTNGYTRYADSVKGRFTISADTSKNTAYLQMNSLRAEDTAVYYCSRWGGDGFYAMDYWGQGTLVTVSSASTKGPSVFPLAPSSKSTSGGTAALGCLVKDYFPEPVTVSWNSGALTSGVHTFPAVLQSSGLYSLSSVVTVPSSSLGTQTYICNVNHKPSNTKVDKKVEPPKSCDKTRTCPPCPAPELLGGPSVFLLPPKIKDTLMISRTPEVTCVVVDVSHEDPEVKFNWYVDGVEVHNAKTKPPEEQYNSTLRVISILTVLHQDWLNGKEYKCKVSNKALPLPEEKTISKQKGQPREPQVYTLPPSRDELTKNQVSLTCLVKGFYPSDIAVEWESNGQQENNYKTTPPVLDSDGSFFLYSKLTVDKSRWQQGNVFSCSVMHEALHNHYTQKSLSLSPGK

SEQ ID NO: 55 - protein, 451 aa, synthetic construct
EVQLVESGGGLVQPGGSLRLSCAASGFNIKDTYIHWVRQAPGKGLEWVARIYPTNGYTRYADSVKGRFTISADTSKNTAYLQMNSLRAEDTAVYYCSRWGGDGFYAMDYWGQGTLVTVSSASTKGPSVFPLAPSSKSTSGGTAALGCLVKDYFPEPVTVSWNSGALTSGVHTFPAVLQSSGLYSLSSVVTVPSSSLGTQTYICNVNHKPSNTKVDKKVEPPKSCDKTHTCPPCPAPELLGGPSVFLLPPKIKDTLMISRTPEVTCVVVDVSHEDPEVKFNWYVDGVEVHNAKTKPPEEQYNSTLRVVSILTVLHQDWLNGKEYKCKVSNKALPLPEEKTISKQKGQPREPQVYTLPPSRGELTKNQVSLTCLVKGFYPSDIAVEWESNGQQENNYKTTPPVLDSDGSFFLYSKLTVDKSRWQQGNVFSCSVMHEALHNHYTQKSLSLSPGK

SEQ ID NO: 56 - protein, 214 aa, synthetic construct
DILLTQSPVILSVSPGERVSFSCRASQSIGTNIHWYQQRTNGSPRLLIKYASESISGIPSRFSGSGSGTDFTLSINSVESEDIADYYCQQNNNWPTTFGAGTKLELKRTVAAPSVFIFPPSDEQLKSGTASVVCLLNNFYPREAKVQWKVDNALQSGNSQESVTEQDSKDSTYSLSSTLTLSKADYEKHKVYACEVTHQGLSSPVTKSFNRGEC

SEQ ID NO: 57 - protein, 449 aa, synthetic construct
QVQLKQSGPGLVQPSQSLSITCTVSGFSLTNYGVHWVRQSPGKGLEWLGVIWSGGNTDYNTPFTSRLSINKDNSKSQVFFKMNSLQSNDTAIYYCARALTYYDYEFAYWGQGTLVTVSAASTKGPSVFPLAPSSKSTSGGTAALGCLVKDYFPEPVTVSWNSGALTSGVHTFPAVLQSSGLYSLSSVVTVPSSSLGTQTYICNVNHKPSNTKVDKKVEPKSCDKTHTCPPCPAPELLGGPSVFLFPPKPKDTLMISRTPEVTCVVVDVSHEDPEVKFNWYVDGVEVHNAKTKPREEQYNSTYRVVSVLTVLHQDWLNGKEYKCKVSNKALPAPIEKTISKAKGQPREPQVYTLPPSRDELTKNQVSLTCLVKGFYPSDIAVEWESNGQPENNYKTTPPVLDSDGSFFLYSKLTVDKSRWQQGNVFSCSVMHEALHNHYTQKSLSLSPGK

SEQ ID NO: 58 - protein, 449 aa, synthetic construct
QVQLKQSGPGLVQPSQSLSITCTVSGFSLTNYGVHWVRQSPGKGLEWLGVIWSGGNTDYNTPFTSRLSINKDNSKSQVFFKMNSLQSNDTAIYYCARALTYYDYEFAYWGQGTLVTVSAASTKGPSVFPLAPSSKSTSGGTAALGCLVKDYFPEPVTVSWNSGALTSGVHTFPAVLQSSGLYSLSSVVTVPSSSLGTQTYICNVNHKPSNTKVDKKVEPKSCDKTHTCPPCPAPELLGGPSVFLLPPKIKDTLMISRTPEVTCVVVDVSHEDPEVKFNWYVDGVEVHNAKTKPPEEQYNSTLRVVSILTVLHQDWLNGKEYKCKVSNKALPLPEEKTISKQKGQPREPQVYTLPPSRDELTKNQVSLTCLVKGFYPSDIAVEWESNGQQENNYKTTPPVLDSDGSFFLYSKLTVDKSRWQQGNVFSCSVMHEALHNHYTQKSLSLSPGK

SEQ ID NO: 59 - protein, 449 aa, synthetic construct
QVQLKQSGPGLVQPSQSLSITCTVSGFSLTNYGVHWVRQSPGKGLEWLGVIWSGGNTDYNTPFTSRLSINKDNSKSQVFFKMNSLQSNDTAIYYCARALTYYDYEFAYWGQGTLVTVSAASTKGPSVFPLAPSSKSTSGGTAALGCLVKDYFPEPVTVSWNSGALTSGVHTFPAVLQSSGLYSLSSVVTVPSSSLGTQTYICNVNHKPSNTKVDKKVEPKSCDKTRTCPPCPAPELLGGPSVFLLPPKIKDTLMISRTPEVTCVVVDVSHEDPEVKFNWYVDGVEVHNAKTKPPEEQYNSTLRVISILTVLHQDWLNGKEYKCKVSNKALPLPEEKTISKQKGQPREPQVYTLPPSRDELTKNQVSLTCLVKGFYPSDIAVEWESNGQQENNYKTTPPVLDSDGSFFLYSKLTVDKSRWQQGNVFSCSVMHEALHNHYTQKSLSLSPGK

SEQ ID NO: 60 - protein, 449 aa, synthetic construct
QVQLKQSGPGLVQPSQSLSITCTVSGFSLTNYGVHWVRQSPGKGLEWLGVIWSGGNTDYNTPFTSRLSINKDNSKSQVFFKMNSLQSNDTAIYYCARALTYYDYEFAYWGQGTLVTVSAASTKGPSVFPLAPSSKSTSGGTAALGCLVKDYFPEPVTVSWNSGALTSGVHTFPAVLQSSGLYSLSSVVTVPSSSLGTQTYICNVNHKPSNTKVDKKVEPKSCDKTHTCPPCPAPELLGGPSVFLLPPKIKDTLMISRTPEVTCVVVDVSHEDPEVKFNWYVDGVEVHNAKTKPPEEQYNSTLRVVSILTVLHQDWLNGKEYKCKVSNKALPLPEEKTISKQKGQPREPQVYTLPPSRGELTKNQVSLTCLVKGFYPSDIAVEWESNGQQENNYKTTPPVLDSDGSFFLYSKLTVDKSRWQQGNVFSCSVMHEALHNHYTQKSLSLSPGK

SEQ ID NO: 61 - protein, 213 aa, synthetic construct
QIVLSQSPAILSASPGEKVTMTCRASSSVSYIHWFQQKPGSSPKPWIYATSNLASGVPVRFSGSGSGTSYSLTISRVEAEDAATYYCQQWTSNPPTFGGGTKLEIKRTVAAPSVFIFPPSDEQLKSGTASVVCLLNNFYPREAKVQWKVDNALQSGNSQESVTEQDSKDSTYSLSSTLTLSKADYEKHKVYACEVTHQGLSSPVTKSFNRGEC

SEQ ID NO: 62 - protein, 451 aa, synthetic construct
QVQLQQPGAELVKPGASVKMSCKASGYTFTSYNMHWVKQTPGRGLEWIGAIYPGNGDTSYNQKFKGKATLTADKSSSTAYMQLSSLTSEDSAVYYCARSTYYGGDWYFNVWGAGTTVTVSAASTKGPSVFPLAPSSKSTSGGTAALGCLVKDYFPEPVTVSWNSGALTSGVHTFPAVLQSSGLYSLSSVVTVPSSSLGTQTYICNVNHKPSNTKVDKKAEPKSCDKTHTCPPCPAPELLGGPSVFLFPPKPKDTLMISRTPEVTCVVVDVSHEDPEVKFNWYVDGVEVHNAKTKPREEQYNSTYRVVSVLTVLHQDWLNGKEYKCKVSNKALPAPIEKTISKAKGQPREPQVYTLPPSRDELTKNQVSLTCLVKGFYPSDIAVEWESNGQPENNYKTTPPVLDSDGSFFLYSKLTVDKSRWQQGNVFSCSVMHEALHNHYTQKSLSLSPGK

SEQ ID NO: 63 - protein, 451 aa, synthetic construct
QVQLQQPGAELVKPGASVKMSCKASGYTFTSYNMHWVKQTPGRGLEWIGAIYPGNGDTSYNQKFKGKATLTADKSSSTAYMQLSSLTSEDSAVYYCARSTYYGGDWYFNVWGAGTTVTVSAASTKGPSVFPLAPSSKSTSGGTAALGCLVKDYFPEPVTVSWNSGALTSGVHTFPAVLQSSGLYSLSSVVTVPSSSLGTQTYICNVNHKPSNTKVDKKAEPKSCDKTHTCPPCPAPELLGGPSVFLLPPKIKDTLMISRTPEVTCVVVDVSHEDPEVKFNWYVDGVEVHNAKTKPPEEQYNSTLRVVSILTVLHQDWLNGKEYKCKVSNKALPLPEEKTISKQKGQPREPQVYTLPPSRDELTKNQVSLTCLVKGFYPSDIAVEWESNGQQENNYKTTPPVLDSDGSFFLYSKLTVDKSRWQQGNVFSCSVMHEALHNHYTQKSLSLSPGK

SEQ ID NO: 64 - protein, 451 aa, synthetic construct
QVQLQQPGAELVKPGASVKMSCKASGYTFTSYNMHWVKQTPGRGLEWIGAIYPGNGDTSYNQKFKGKATLTADKSSSTAYMQLSSLTSEDSAVYYCARSTYYGGDWYFNVWGAGTTVTVSAASTKGPSVFPLAPSSKSTSGGTAALGCLVKDYFPEPVTVSWNSGALTSGVHTFPAVLQSSGLYSLSSVVTVPSSSLGTQTYICNVNHKPSNTKVDKKAEPKSCDKTRTCPPCPAPELLGGPSVFLLPPKIKDTLMISRTPEVTCVVVDVSHEDPEVKFNWYVDGVEVHNAKTKPPEEQYNSTLRVISILTVLHQDWLNGKEYKCKVSNKALPLPEEKTISKQKGQPREPQVYTLPPSRDELTKNQVSLTCLVKGFYPSDIAVEWESNGQQENNYKTTPPVLDSDGSFFLYSKLTVDKSRWQQGNVFSCSVMHEALHNHYTQKSLSLSPGK

SEQ ID NO: 65 - protein, 451 aa, synthetic construct
QVQLQQPGAELVKPGASVKMSCKASGYTFTSYNMHWVKQTPGRGLEWIGAIYPGNGDTSYNQKFKGKATLTADKSSSTAYMQLSSLTSEDSAVYYCARSTYYGGDWYFNVWGAGTTVTVSAASTKGPSVFPLAPSSKSTSGGTAALGCLVKDYFPEPVTVSWNSGALTSGVHTFPAVLQSSGLYSLSSVVTVPSSSLGTQTYICNVNHKPSNTKVDKKAEPKSCDKTHTCPPCPAPELLGGPSVFLLPPKIKDTLMISRTPEVTCVVVDVSHEDPEVKFNWYVDGVEVHNAKTKPPEEQYNSTLRVVSILTVLHQDWLNGKEYKCKVSNKALPLPEEKTISKQKGQPREPQVYTLPPSRGELTKNQVSLTCLVKGFYPSDIAVEWESNGQQENNYKTTPPVLDSDGSFFLYSKLTVDKSRWQQGNVFSCSVMHEALHNHYTQKSLSLSPGK